European Patent Specification EP 3 462 883 B1, published August 16, 2023. Title: COMPOSITIONS AND METHODS FOR TREATING CANCER. Applicant: THE PACIFIC HEART, LUNG & BLOOD INSTITUTE. The sequence listing filed with the application follows.

SEQUENCE LISTING (13 sequences)

SEQ ID NO: 1 - protein, 536 aa, Homo sapiens
MCHQQLVISWFSLVFLASPLVAIWELKKDVYVVELDWYPDAPGEMVVLTCDTPEEDGITWTLDQSSEVLGSGKTLTIQVKEFGDAGQYTCHKGGEVLSHSLLLLHKKEDGIWSTDILKDQKEPKNKTFLRCEAKNYSGRFTCWWLTTISTDLTFSVKSSRGSSDPQGVTCGAATLSAERVRGDNKEYEYSVECQEDSACPAAEESLPIEVMVDAVHKLKYENYTSSFFIRDIIKPDPPKNLQLKPLKNSRQVEVSWEYPDTWSTPHSYFSLTFCVQVQGKSKREKKDRVFTDKTSATVICRKNASISVRAQDRYYSSSWSEWASVPCSVPGVGVPGVGARNLPVATPDPGMFPCLHHSQNLLRAVSNMLQKARQTLEFYPCTSEEIDHEDITKDKTSTVEACLPLELTKNESCLNSRETSFITNGSCLASRKTSFMMALCLSSIYEDLKMYQVEFKTMNAKLLMDPKRQIFLDQNMLAVIDELMQALNFNSETVPQKSSLEEPDFYKTKIKLCILLHAFRIRAVTIDRVMSYLNAS

SEQ ID NO: 2 - protein, 397 aa, Artificial Sequence
  Description of Artificial Sequence: Synthetic polypeptide
TFPKRGQTCVVHYTGMLEDGKKVDSSRDRNKPFKFMLGKQEVIRGWEEGVAQMSVGQRAKLTISPDYAYGATGHPGIIPPHATLVFDVELLKLESGGGSGVDGFGDVGALESLRGNADLAYILSMEPCGHCLIINNVNFCRESGLRTRTGSNIDCEKLRRRFSSLHFMVEVKGDLTAKKMVLALLELAQQDHGALDCCVVVILSHGCQASHLQFPGAVYGTDGCPVSVEKIVNIFNGTSCPSLGGKPKLFFIQACGGEQKDHGFEVASTSPEDESPGSNPEPDATPFQEGLRTFDQLDAISSLPTPSDIFVSYSTFPGFVSWRDPKSGSWYVETLDDIFEQWAHSEDLQSLLLRVANAVSVKGIYKQMPGCFNFLRKKLFFKTSVDYPYDVPDYALD

SEQ ID NO: 3 - protein, 413 aa, Artificial Sequence
  Description of Artificial Sequence: Synthetic polypeptide
MLEGVQVETISPGDGRTFPKRGQTCVVHYTGMLEDGKKVDSSRDRNKPFKFMLGKQEVIRGWEEGVAQMSVGQRAKLTISPDYAYGATGHPGIIPPHATLVFDVELLKLESGGGSGVDGFGDVGALESLRGNADLAYILSMEPCGHCLIINNVNFCRESGLRTRTGSNIDCEKLRRRFSSLHFMVEVKGDLTAKKMVLALLELAQQDHGALDCCVVVILSHGCQASHLQFPGAVYGTDGCPVSVEKIVNIFNGTSCPSLGGKPKLFFIQACGGEQKDHGFEVASTSPEDESPGSNPEPDATPFQEGLRTFDQLDAISSLPTPSDIFVSYSTFPGFVSWRDPKSGSWYVETLDDIFEQWAHSEDLQSLLLRVANAVSVKGIYKQMPGCFNFLRKKLFFKTSVDYPYDVPDYALD

SEQ ID NO: 4 - protein, 328 aa, Homo sapiens
MCHQQLVISWFSLVFLASPLVAIWELKKDVYVVELDWYPDAPGEMVVLTCDTPEEDGITWTLDQSSEVLGSGKTLTIQVKEFGDAGQYTCHKGGEVLSHSLLLLHKKEDGIWSTDILKDQKEPKNKTFLRCEAKNYSGRFTCWWLTTISTDLTFSVKSSRGSSDPQGVTCGAATLSAERVRGDNKEYEYSVECQEDSACPAAEESLPIEVMVDAVHKLKYENYTSSFFIRDIIKPDPPKNLQLKPLKNSRQVEVSWEYPDTWSTPHSYFSLTFCVQVQGKSKREKKDRVFTDKTSATVICRKNASISVRAQDRYYSSSWSEWASVPCS

SEQ ID NO: 5 - protein, 253 aa, Homo sapiens
MWPPGSASQPPPSPAAATGLHPAARPVSLQCRLSMCPARSLLLVATLVLLDHLSLARNLPVATPDPGMFPCLHHSQNLLRAVSNMLQKARQTLEFYPCTSEEIDHEDITKDKTSTVEACLPLELTKNESCLNSRETSFITNGSCLASRKTSFMMALCLSSIYEDLKMYQVEFKTMNAKLLMDPKRQIFLDQNMLAVIDELMQALNFNSETVPQKSSLEEPDFYKTKIKLCILLHAFRIRAVTIDRVMSYLNAS

SEQ ID NO: 6 - protein, 285 aa, Homo sapiens
GSGGFGDVGALESLRGNADLAYILSMEPCGHCLIINNVNFCRESGLRTRTGSNIDCEKLRRRFSSLHFMVEVKGDLTAKKMVLALLELAQQDHGALDCCVVVILSHGCQASHLQFPGAVYGTDGCPVSVEKIVNIFNGTSCPSLGGKPKLFFIQACGGEQKDHGFEVASTSPEDESPGSNPEPDATPFQEGLRTFDQLDAISSLPTPSDIFVSYSTFPGFVSWRDPKSGSWYVETLDDIFEQWAHSEDLQSLLLRVANAVSVKGIYKQMPGCFNFLRKKLFFKTS

SEQ ID NO: 7 - protein, 5 aa, Artificial Sequence
  Description of Artificial Sequence: Synthetic peptide
EFLID

SEQ ID NO: 8 - protein, 15 aa, Artificial Sequence
  Description of Artificial Sequence: Synthetic peptide
PDPDMIRYIDEFGQT

SEQ ID NO: 9 - protein, 8 aa, Artificial Sequence
  Description of Artificial Sequence: Synthetic peptide
GGGGGGGG

SEQ ID NO: 10 - protein, 6 aa, Artificial Sequence
  Description of Artificial Sequence: Synthetic peptide
GGGGGG

SEQ ID NO: 11 - protein, 15 aa, Artificial Sequence
  Description of Artificial Sequence: Synthetic peptide
GGGGSGGGGSGGGGS

SEQ ID NO: 12 - protein, 5 aa, Artificial Sequence
  Description of Artificial Sequence: Synthetic peptide
EAAAK

SEQ ID NO: 13 - protein, 6 aa, Artificial Sequence
  Description of Artificial Sequence: Synthetic 6xHis tag
HHHHHH